European Patent Specification EP 3 356 552 B1, published March 19, 2025. Title: HIGH-MOLECULAR WEIGHT DNA SAMPLE TRACKING TAGS FOR NEXT GENERATION SEQUENCING. Applicant: Kapa Biosystems, Inc. Ranik, Martin van der Walt, Eric McEwan, Paul. The sequence listing filed with the application follows.

SEQUENCE LISTING (107 sequences)

SEQ ID NO: 1 - DNA, 60 bp, Artificial Sequence
  synthetic nucleic acid
atgcacaaggccgacaataggcacgagcatagaagttagtacgtagcgtggtcgcataag

SEQ ID NO: 2 - DNA, 19 bp, Artificial Sequence
  synthetic nucleic acid
atgcacaaggccgacaata

SEQ ID NO: 3 - DNA, 22 bp, Artificial Sequence
  synthetic nucleic acid
ggcacgagcatagaagttagta

SEQ ID NO: 4 - DNA, 19 bp, Artificial Sequence
  synthetic nucleic acid
cgtagcgtggtcgcataag

SEQ ID NO: 5 - DNA, 60 bp, Artificial Sequence
  synthetic nucleic acid
atgcacaaggccgacaatagagtaggacaatgattgagaagcgtagcgtggtcgcataag

SEQ ID NO: 6 - DNA, 22 bp, Artificial Sequence
  synthetic nucleic acid
gagtaggacaatgattgagaag

SEQ ID NO: 7 - DNA, 20 bp, Artificial Sequence
  synthetic nucleic acid
ccttgtgcatcttatgcgac

SEQ ID NO: 8 - DNA, 19 bp, Artificial Sequence
  synthetic nucleic acid
atgcacaaggccgacaata

SEQ ID NO: 9 - DNA, 19 bp, Artificial Sequence
  synthetic nucleic acid
cttatgcgaccacgctacg

SEQ ID NO: 10 - DNA, 120 bp, Artificial Sequence
  synthetic nucleic acid
cttatgcgaccacgctacgtactaacttctatgctcgtgcctattgtcggccttgtgcatcttatgcgaccacgctacgtactaacttctatgctcgtgcctattgtcggccttgtgcat

SEQ ID NO: 11 - DNA, 60 bp, Artificial Sequence
  synthetic nucleic acid
atgcacaaggccgacaataactttgagcaaacgtcgtctgtcgtagcgtggtcgcataag

SEQ ID NO: 12 - DNA, 60 bp, Artificial Sequence
  synthetic nucleic acid
atgcacaaggccgacaatataagcaccttctgtgcgtaatgcgtagcgtggtcgcataag

SEQ ID NO: 13 - DNA, 60 bp, Artificial Sequence
  synthetic nucleic acid
atgcacaaggccgacaatattacgacgtagctccgatttagcgtagcgtggtcgcataag

SEQ ID NO: 14 - DNA, 60 bp, Artificial Sequence
  synthetic nucleic acid
atgcacaaggccgacaataagtgagactgatccttctagctcgtagcgtggtcgcataag

SEQ ID NO: 15 - DNA, 60 bp, Artificial Sequence
  synthetic nucleic acid
atgcacaaggccgacaatactctgattcgaatgcaagtcgtcgtagcgtggtcgcataag

SEQ ID NO: 16 - DNA, 60 bp, Artificial Sequence
  synthetic nucleic acid
atgcacaaggccgacaataggtagcatcaatttagctcgtccgtagcgtggtcgcataag

SEQ ID NO: 17 - DNA, 60 bp, Artificial Sequence
  synthetic nucleic acid
atgcacaaggccgacaatacacggctatttcacgttgtagacgtagcgtggtcgcataag

SEQ ID NO: 18 - DNA, 60 bp, Artificial Sequence
  synthetic nucleic acid
atgcacaaggccgacaatagccggaactcttttaaggcattcgtagcgtggtcgcataag

SEQ ID NO: 19 - DNA, 60 bp, Artificial Sequence
  synthetic nucleic acid
atgcacaaggccgacaatagcgccaattatgtggactacttcgtagcgtggtcgcataag

SEQ ID NO: 20 - DNA, 60 bp, Artificial Sequence
  synthetic nucleic acid
atgcacaaggccgacaatacgtcacctgtagaaatgtcgttcgtagcgtggtcgcataag

SEQ ID NO: 21 - DNA, 60 bp, Artificial Sequence
  synthetic nucleic acid
atgcacaaggccgacaatagagcaggtcctatcattatctgcgtagcgtggtcgcataag

SEQ ID NO: 22 - DNA, 60 bp, Artificial Sequence
  synthetic nucleic acid
atgcacaaggccgacaatatcattcatcgattggcaggtaccgtagcgtggtcgcataag

SEQ ID NO: 23 - DNA, 60 bp, Artificial Sequence
  synthetic nucleic acid
atgcacaaggccgacaatatcgctgagacggttctaaatctcgtagcgtggtcgcataag

SEQ ID NO: 24 - DNA, 60 bp, Artificial Sequence
  synthetic nucleic acid
atgcacaaggccgacaatacattgacgggttagatatcctccgtagcgtggtcgcataag

SEQ ID NO: 25 - DNA, 18 bp, Artificial Sequence
  T7 RNA polymerase promoter sequence
taatacgactcactatag

SEQ ID NO: 26 - DNA, 17 bp, Artificial Sequence
  synthetic nucleic acid
gtagcgtggtcgcataa

SEQ ID NO: 27 - DNA, 59 bp, Artificial Sequence
  synthetic nucleic acid
taatacgactcactatagggcacgagcatagaagttagtacgtagcgtggtcgcataag

SEQ ID NO: 28 - DNA, 58 bp, Artificial Sequence
  synthetic nucleic acid
atgcacaaggccgacaataatcgcactgtagtggtagtgcgtagcgtggtcgcataag

SEQ ID NO: 29 - DNA, 58 bp, Artificial Sequence
  synthetic nucleic acid
atgcacaaggccgacaataatcatgcgaggctctctctacgtagcgtggtcgcataag

SEQ ID NO: 30 - DNA, 58 bp, Artificial Sequence
  synthetic nucleic acid
atgcacaaggccgacaataccatagtccggtctctgtatcgtagcgtggtcgcataag

SEQ ID NO: 31 - DNA, 58 bp, Artificial Sequence
  synthetic nucleic acid
atgcacaaggccgacaatatcgcatcaagaggctccaatcgtagcgtggtcgcataag

SEQ ID NO: 32 - DNA, 58 bp, Artificial Sequence
  synthetic nucleic acid
atgcacaaggccgacaatagagatatcaacttcgcgagccgtagcgtggtcgcataag

SEQ ID NO: 33 - DNA, 58 bp, Artificial Sequence
  synthetic nucleic acid
atgcacaaggccgacaatacgcgaattagaactagtccgcgtagcgtggtcgcataag

SEQ ID NO: 34 - DNA, 58 bp, Artificial Sequence
  synthetic nucleic acid
atgcacaaggccgacaataagtaggacctgcgttaagctcgtagcgtggtcgcataag

SEQ ID NO: 35 - DNA, 58 bp, Artificial Sequence
  synthetic nucleic acid
atgcacaaggccgacaatactcgccagtatacaactgctcgtagcgtggtcgcataag

SEQ ID NO: 36 - DNA, 58 bp, Artificial Sequence
  synthetic nucleic acid
atgcacaaggccgacaataactcgtcctctagatgcagacgtagcgtggtcgcataag

SEQ ID NO: 37 - DNA, 58 bp, Artificial Sequence
  synthetic nucleic acid
atgcacaaggccgacaatagagaagtacggcgcgaattacgtagcgtggtcgcataag

SEQ ID NO: 38 - DNA, 58 bp, Artificial Sequence
  synthetic nucleic acid
atgcacaaggccgacaatagctgctatgcactatctctccgtagcgtggtcgcataag

SEQ ID NO: 39 - DNA, 58 bp, Artificial Sequence
  synthetic nucleic acid
atgcacaaggccgacaataatgtcgcactacaggttgcacgtagcgtggtcgcataag

SEQ ID NO: 40 - DNA, 58 bp, Artificial Sequence
  synthetic nucleic acid
atgcacaaggccgacaatatatcacctatccacatggcccgtagcgtggtcgcataag

SEQ ID NO: 41 - DNA, 58 bp, Artificial Sequence
  synthetic nucleic acid
atgcacaaggccgacaatatcacctgtactgtggtggttcgtagcgtggtcgcataag

SEQ ID NO: 42 - DNA, 58 bp, Artificial Sequence
  synthetic nucleic acid
atgcacaaggccgacaatagatcgcatatagtgcacctgcgtagcgtggtcgcataag

SEQ ID NO: 43 - DNA, 58 bp, Artificial Sequence
  synthetic nucleic acid
atgcacaaggccgacaatacttaacggttgcacggattccgtagcgtggtcgcataag

SEQ ID NO: 44 - DNA, 58 bp, Artificial Sequence
  synthetic nucleic acid
atgcacaaggccgacaatacacaggctgtctaatctacgcgtagcgtggtcgcataag

SEQ ID NO: 45 - DNA, 58 bp, Artificial Sequence
  synthetic nucleic acid
atgcacaaggccgacaatacctatagcgcaattgtgtcccgtagcgtggtcgcataag

SEQ ID NO: 46 - DNA, 58 bp, Artificial Sequence
  synthetic nucleic acid
atgcacaaggccgacaatacctgtagcatgcaatgacgtcgtagcgtggtcgcataag

SEQ ID NO: 47 - DNA, 58 bp, Artificial Sequence
  synthetic nucleic acid
atgcacaaggccgacaatagcgtgtgattaaccttgcagcgtagcgtggtcgcataag

SEQ ID NO: 48 - DNA, 58 bp, Artificial Sequence
  synthetic nucleic acid
atgcacaaggccgacaatatagttcataggtccgtgacgcgtagcgtggtcgcataag

SEQ ID NO: 49 - DNA, 58 bp, Artificial Sequence
  synthetic nucleic acid
atgcacaaggccgacaataggtctattcggagcacgttacgtagcgtggtcgcataag

SEQ ID NO: 50 - DNA, 58 bp, Artificial Sequence
  synthetic nucleic acid
atgcacaaggccgacaatacttaggctaggaggcttgtacgtagcgtggtcgcataag

SEQ ID NO: 51 - DNA, 58 bp, Artificial Sequence
  synthetic nucleic acid
atgcacaaggccgacaatactaacgtggttagtgagcaccgtagcgtggtcgcataag

SEQ ID NO: 52 - DNA, 58 bp, Artificial Sequence
  synthetic nucleic acid
atgcacaaggccgacaataggtctaagaagtcatctgcgcgtagcgtggtcgcataag

SEQ ID NO: 53 - DNA, 58 bp, Artificial Sequence
  synthetic nucleic acid
atgcacaaggccgacaataccaatgtagccgctattaggcgtagcgtggtcgcataag

SEQ ID NO: 54 - DNA, 58 bp, Artificial Sequence
  synthetic nucleic acid
atgcacaaggccgacaatactgtgtattacggagccaagcgtagcgtggtcgcataag

SEQ ID NO: 55 - DNA, 58 bp, Artificial Sequence
  synthetic nucleic acid
atgcacaaggccgacaataaccggtggtgatcagttaagcgtagcgtggtcgcataag

SEQ ID NO: 56 - DNA, 58 bp, Artificial Sequence
  synthetic nucleic acid
atgcacaaggccgacaatattcacggtatgcacaccttgcgtagcgtggtcgcataag

SEQ ID NO: 57 - DNA, 58 bp, Artificial Sequence
  synthetic nucleic acid
atgcacaaggccgacaatacgtatgacctcacactctcacgtagcgtggtcgcataag

SEQ ID NO: 58 - DNA, 58 bp, Artificial Sequence
  synthetic nucleic acid
atgcacaaggccgacaataaactggcgccgaacatctaacgtagcgtggtcgcataag

SEQ ID NO: 59 - DNA, 58 bp, Artificial Sequence
  synthetic nucleic acid
atgcacaaggccgacaatagatcggtcgcactaatgaaccgtagcgtggtcgcataag

SEQ ID NO: 60 - DNA, 58 bp, Artificial Sequence
  synthetic nucleic acid
atgcacaaggccgacaatagtctgaacacgtgaatcggacgtagcgtggtcgcataag

SEQ ID NO: 61 - DNA, 58 bp, Artificial Sequence
  synthetic nucleic acid
atgcacaaggccgacaatattcctcgatgctatcgcacacgtagcgtggtcgcataag

SEQ ID NO: 62 - DNA, 58 bp, Artificial Sequence
  synthetic nucleic acid
atgcacaaggccgacaataagattacgaaccgtaggacccgtagcgtggtcgcataag

SEQ ID NO: 63 - DNA, 58 bp, Artificial Sequence
  synthetic nucleic acid
atgcacaaggccgacaatacatgttcgtattggtgcctgcgtagcgtggtcgcataag

SEQ ID NO: 64 - DNA, 58 bp, Artificial Sequence
  synthetic nucleic acid
atgcacaaggccgacaatagcctgtgttccatcagcttacgtagcgtggtcgcataag

SEQ ID NO: 65 - DNA, 58 bp, Artificial Sequence
  synthetic nucleic acid
atgcacaaggccgacaataaaggtcgtgagtactccttccgtagcgtggtcgcataag

SEQ ID NO: 66 - DNA, 58 bp, Artificial Sequence
  synthetic nucleic acid
atgcacaaggccgacaataagtgtattggcgaaccgactcgtagcgtggtcgcataag

SEQ ID NO: 67 - DNA, 58 bp, Artificial Sequence
  synthetic nucleic acid
atgcacaaggccgacaatagcctcgatgtatattgcgcacgtagcgtggtcgcataag

SEQ ID NO: 68 - DNA, 58 bp, Artificial Sequence
  synthetic nucleic acid
atgcacaaggccgacaatacgctagaatgaggtaggcaacgtagcgtggtcgcataag

SEQ ID NO: 69 - DNA, 58 bp, Artificial Sequence
  synthetic nucleic acid
atgcacaaggccgacaatacatacgccttagtcggaacacgtagcgtggtcgcataag

SEQ ID NO: 70 - DNA, 58 bp, Artificial Sequence
  synthetic nucleic acid
atgcacaaggccgacaatattgcttacgatctgcgtaggcgtagcgtggtcgcataag

SEQ ID NO: 71 - DNA, 58 bp, Artificial Sequence
  synthetic nucleic acid
atgcacaaggccgacaatatgcgttattgcagtatcgcccgtagcgtggtcgcataag

SEQ ID NO: 72 - DNA, 58 bp, Artificial Sequence
  synthetic nucleic acid
atgcacaaggccgacaatactagacgcctgaagaatggacgtagcgtggtcgcataag

SEQ ID NO: 73 - DNA, 58 bp, Artificial Sequence
  synthetic nucleic acid
atgcacaaggccgacaatagagaaggaacgagtgttacccgtagcgtggtcgcataag

SEQ ID NO: 74 - DNA, 58 bp, Artificial Sequence
  synthetic nucleic acid
atgcacaaggccgacaataattcaaccgactcgaactgccgtagcgtggtcgcataag

SEQ ID NO: 75 - DNA, 58 bp, Artificial Sequence
  synthetic nucleic acid
atgcacaaggccgacaatagtactcctagatatgacggccgtagcgtggtcgcataag

SEQ ID NO: 76 - DNA, 58 bp, Artificial Sequence
  synthetic nucleic acid
atgcacaaggccgacaatacgcggacatagttaagcgtacgtagcgtggtcgcataag

SEQ ID NO: 77 - DNA, 58 bp, Artificial Sequence
  synthetic nucleic acid
atgcacaaggccgacaatattcgtacgagacgtgctgatcgtagcgtggtcgcataag

SEQ ID NO: 78 - DNA, 58 bp, Artificial Sequence
  synthetic nucleic acid
atgcacaaggccgacaataacacataacgccgcaatctccgtagcgtggtcgcataag

SEQ ID NO: 79 - DNA, 58 bp, Artificial Sequence
  synthetic nucleic acid
atgcacaaggccgacaatatagaccagcctactattcgccgtagcgtggtcgcataag

SEQ ID NO: 80 - DNA, 58 bp, Artificial Sequence
  synthetic nucleic acid
atgcacaaggccgacaatagacacagtgtctctaatgcccgtagcgtggtcgcataag

SEQ ID NO: 81 - DNA, 58 bp, Artificial Sequence
  synthetic nucleic acid
atgcacaaggccgacaataatggctcgcaggagatgtatcgtagcgtggtcgcataag

SEQ ID NO: 82 - DNA, 58 bp, Artificial Sequence
  synthetic nucleic acid
atgcacaaggccgacaatagcttacggtgtgatagtacgcgtagcgtggtcgcataag

SEQ ID NO: 83 - DNA, 58 bp, Artificial Sequence
  synthetic nucleic acid
atgcacaaggccgacaatatgtactacggctgattcctccgtagcgtggtcgcataag

SEQ ID NO: 84 - DNA, 58 bp, Artificial Sequence
  synthetic nucleic acid
atgcacaaggccgacaatatcgttctgtactggttgctccgtagcgtggtcgcataag

SEQ ID NO: 85 - DNA, 58 bp, Artificial Sequence
  synthetic nucleic acid
atgcacaaggccgacaatatgagacggtatgtcgcagatcgtagcgtggtcgcataag

SEQ ID NO: 86 - DNA, 58 bp, Artificial Sequence
  synthetic nucleic acid
atgcacaaggccgacaataaccttgcaatccgtcacaagcgtagcgtggtcgcataag

SEQ ID NO: 87 - DNA, 58 bp, Artificial Sequence
  synthetic nucleic acid
atgcacaaggccgacaataaccaagagtcttgtccagagcgtagcgtggtcgcataag

SEQ ID NO: 88 - DNA, 58 bp, Artificial Sequence
  synthetic nucleic acid
atgcacaaggccgacaataggtaagctgacattcgacaccgtagcgtggtcgcataag

SEQ ID NO: 89 - DNA, 58 bp, Artificial Sequence
  synthetic nucleic acid
atgcacaaggccgacaatacaattgaggtgtgcaatggccgtagcgtggtcgcataag

SEQ ID NO: 90 - DNA, 58 bp, Artificial Sequence
  synthetic nucleic acid
atgcacaaggccgacaataggctgttcgtgataggatcacgtagcgtggtcgcataag

SEQ ID NO: 91 - DNA, 58 bp, Artificial Sequence
  synthetic nucleic acid
atgcacaaggccgacaataaggcggtgcgtaatagtgttcgtagcgtggtcgcataag

SEQ ID NO: 92 - DNA, 58 bp, Artificial Sequence
  synthetic nucleic acid
atgcacaaggccgacaatagatacgaagttacagcctgccgtagcgtggtcgcataag

SEQ ID NO: 93 - DNA, 58 bp, Artificial Sequence
  synthetic nucleic acid
atgcacaaggccgacaatactaatgcatactgctggaggcgtagcgtggtcgcataag

SEQ ID NO: 94 - DNA, 58 bp, Artificial Sequence
  synthetic nucleic acid
atgcacaaggccgacaatagcttcggttagactagagagcgtagcgtggtcgcataag

SEQ ID NO: 95 - DNA, 58 bp, Artificial Sequence
  synthetic nucleic acid
atgcacaaggccgacaataccggttgatattctaggccacgtagcgtggtcgcataag

SEQ ID NO: 96 - DNA, 58 bp, Artificial Sequence
  synthetic nucleic acid
atgcacaaggccgacaatacatgaggagaggtattcctccgtagcgtggtcgcataag

SEQ ID NO: 97 - DNA, 58 bp, Artificial Sequence
  synthetic nucleic acid
atgcacaaggccgacaatagaatcgtctacctagctcgtcgtagcgtggtcgcataag

SEQ ID NO: 98 - DNA, 58 bp, Artificial Sequence
  synthetic nucleic acid
atgcacaaggccgacaataggtgaagttagacctggactcgtagcgtggtcgcataag

SEQ ID NO: 99 - DNA, 58 bp, Artificial Sequence
  synthetic nucleic acid
atgcacaaggccgacaataggattgtaggatgactcctgcgtagcgtggtcgcataag

SEQ ID NO: 100 - DNA, 58 bp, Artificial Sequence
  synthetic nucleic acid
atgcacaaggccgacaataagattgcgccggtacaattgcgtagcgtggtcgcataag

SEQ ID NO: 101 - DNA, 58 bp, Artificial Sequence
  synthetic nucleic acid
atgcacaaggccgacaatagttccgccgagtattcatagcgtagcgtggtcgcataag

SEQ ID NO: 102 - DNA, 58 bp, Artificial Sequence
  synthetic nucleic acid
atgcacaaggccgacaatacttgtacagcagtctaagcccgtagcgtggtcgcataag

SEQ ID NO: 103 - DNA, 58 bp, Artificial Sequence
  synthetic nucleic acid
atgcacaaggccgacaatagaagcgcgcatgaattgatccgtagcgtggtcgcataag

SEQ ID NO: 104 - DNA, 58 bp, Artificial Sequence
  synthetic nucleic acid
atgcacaaggccgacaatataccggaatcgtgtctgtctcgtagcgtggtcgcataag

SEQ ID NO: 105 - DNA, 58 bp, Artificial Sequence
  synthetic nucleic acid
atgcacaaggccgacaatagcttcatggcaatgcatcgtcgtagcgtggtcgcataag

SEQ ID NO: 106 - DNA, 58 bp, Artificial Sequence
  synthetic nucleic acid
atgcacaaggccgacaatagacctgcgtaccttgtcttacgtagcgtggtcgcataag

SEQ ID NO: 107 - DNA, 58 bp, Artificial Sequence
  synthetic nucleic acid
atgcacaaggccgacaatagccgcagattacaaggattgcgtagcgtggtcgcataag